European Patent Application EP 4 190 346 A1, published June 7, 2023. Title: A composition for preventing or treating inflammatory diseases and uses thereof. Applicant: SEOUL NATIONAL UNIVERSITY HOSPITAL. The sequence listing filed with the application follows.

SEQUENCE LISTING (33 sequences)

SEQ ID NO: 1 - DNA, 1737 bp, Artificial Sequence
  Zkscan 8(Zinc finger protein with KRAB and SCAN domains 8)
atggctgaagaatcaagaaagccttcagccccatccccaccagaccagactcctgaagaggatcttgtaatcgtcaaggtagaggaggatcatggttgggaccaggaatctagtctgcatgaaagtaaccctcttggccaagaagtgttccgcctgcgcttcaggcagttacgctaccaggagacactaggaccccgagaagctctgatccaactacgggccctttgccatcagtggctgaggccagatttgaacaccaaggaacagatcctggagctgctggtgctggagcagttcttgaccatcctacctgaggagctccagacactggttaaggaacatcagctagagaacggagaggaggtggtgaccctattagaggatttggaaaggcagattgatatactaggacgaccagtctcagctcgcgtacatggacatagggtactctgggaggaggtagtacattcagcatctgcaccagagcctccaaatactcagctccaatctgaggcaacccaacataaatctccagtgccccaagagtcacaagagagagccatgtctacttcccagagtcctactcgttcccagaaaggaagttctggagaccaggaaatgacagctacacttctcacagcagggttccagactttggagaagattgaagacatggctgtgtcccttattcgagaggagtggcttcttgatccatcacagaaggatctgtgtagagataacaggccagaaaatttcagaaacatgttctccctgggtggtgagaccaggagtgagaacagggaattagcttcaaaacaggtaatatctactggaatccagccacatggagagacagctgccaaatgcaacggggatgttatcaggggtcttgagcatgaagaagcccgagaccttctgggcagattagagaggcagcggggaaatcccacacaagagagacgacataaatgtgatgaatgtgggaaaagctttgctcagagctcaggccttgttcgccactggagaatccacactggggagaaaccctatcagtgtaatgtgtgtggtaaagccttcagttacaggtcagcccttctttcacatcaggatatccacaacaaagtaaaacgctatcactgtaaggagtgtggcaaagccttcagtcagaacacaggcctgattctgcaccagagaatccacactggggagaagccatatcagtgcaatcagtgtgggaaggctttcagtcagagtgcgggccttattctgcaccagagaatccacagtggagagagaccctatgaatgtaatgagtgtgggaaagctttcagtcatagctcacacctcattggacatcagagaatccacactggggagaagccctatgagtgtgatgagtgtgggaaaaccttcaggcggagctcacatcttattggtcatcagaggagccacactggggagaaaccctacaaatgcaatgagtgtgggagggccttcagtcagaagtcaggccttattgaacatcagagaatccacactggagaaagaccctataaatgtaaagaatgtgggaaagctttcaatgggaacactggtctcattcaacacctgagaattcacacaggggagaagccctaccaatgtaatgagtgtgggaaagcctttattcagaggtcaagtctcattcgacatcagagaatccacagtggtgaaaaatctgaatccataagcgtttag

SEQ ID NO: 2 - protein, 578 aa, Artificial Sequence
  Zkscan 8(Zinc finger protein with KRAB and SCAN domains 8)
MAEESRKPSAPSPPDQTPEEDLVIVKVEEDHGWDQESSLHESNPLGQEVFRLRFRQLRYQETLGPREALIQLRALCHQWLRPDLNTKEQILELLVLEQFLTILPEELQTLVKEHQLENGEEVVTLLEDLERQIDILGRPVSARVHGHRVLWEEVVHSASAPEPPNTQLQSEATQHKSPVPQESQERAMSTSQSPTRSQKGSSGDQEMTATLLTAGFQTLEKIEDMAVSLIREEWLLDPSQKDLCRDNRPENFRNMFSLGGETRSENRELASKQVISTGIQPHGETAAKCNGDVIRGLEHEEARDLLGRLERQRGNPTQERRHKCDECGKSFAQSSGLVRHWRIHTGEKPYQCNVCGKAFSYRSALLSHQDIHNKVKRYHCKECGKAFSQNTGLILHQRIHTGEKPYQCNQCGKAFSQSAGLILHQRIHSGERPYECNECGKAFSHSSHLIGHQRIHTGEKPYECDECGKTFRRSSHLIGHQRSHTGEKPYKCNECGRAFSQKSGLIEHQRIHTGERPYKCKECGKAFNGNTGLIQHLRIHTGEKPYQCNECGKAFIQRSSLIRHQRIHSGEKSESISV

SEQ ID NO: 3 - DNA, 1737 bp, Artificial Sequence
  Optimized zkscan8 gene sequence
atggcggaggaaagtcggaaaccatccgcccccagtccgcccgatcaaacccctgaagaagaccttgtcatagtcaaagtcgaggaggaccacggctgggatcaggaaagcagccttcacgagtctaacccgcttggacaagaggtttttcgcctgagatttcgtcagttgcgttaccaggagactcttggtccacgggaagctcttatacaactgagagcattgtgtcaccaatggttgcggccagaccttaatactaaagagcagatattagaactgctggttttggagcaatttttgacaatactgccggaggaactgcaaactcttgtcaaagagcaccaactggaaaatggtgaggaagttgtaacccttcttgaggacctggagagacagattgatatccttggccgcccagtatcagcgcgcgtgcatggccatcgcgtcttgtgggaagaggtcgtccatagcgcaagtgcccctgagccaccaaacactcagcttcagagcgaggcgacacagcataagtcgcctgttcctcaggagagccaggaacgggccatgagtaccagtcagtcgcctacaagaagccaaaagggctctagtggggatcaggaaatgacagccacgttacttaccgcagggttccagaccttagaaaaaatcgaggatatggccgtatcgttgatccgggaagagtggctgcttgacccatctcagaaggatctgtgcagagacaatcggcctgagaacttccgcaatatgttctcccttggtggagaaacgcggtcggaaaatagagagctggcaagcaagcaagttatcagcacaggcatccagcctcatggcgaaacggctgctaaatgtaatggtgatgtcatacgtgggttagaacatgaggaagcccgggatttattggggcgtctggaacgccagcgtggaaatccgacacaggagcggcgtcataaatgcgatgaatgtggtaagagtttcgctcaatcgtctgggcttgttcggcattggcggattcatacgggagagaagccttaccagtgtaatgtatgcgggaaagcgttttcataccggtctgcccttctttcacatcaagatatccataacaaggtcaaacgttatcactgcaaagaatgcggtaaagcgttttctcagaatacggggctgatcttacatcagagaatccataccggagaaaaaccttatcaatgcaatcagtgcggaaaggccttttctcagagcgcagggctgattttgcatcaaagaattcattcaggcgagcgtccctatgagtgtaatgagtgcggcaaagcttttagccacagctcgcacctgattggtcatcaacgcattcacacgggtgaaaagccctatgaatgcgatgagtgcggaaagacgtttcgccgctcgtcgcatttaataggccaccaacgttctcatacaggagaaaaaccgtacaagtgcaatgaatgtgggagagccttcagccagaaaagcggtctgatagagcaccaacgtatccacacgggggagagaccgtacaaatgcaaagaatgtgggaaagcctttaatggaaataccgggctgattcagcacctgagaattcacactggagagaagccttaccaatgtaacgagtgcggtaaagcttttatacaacgttcgagtttaatacgccatcaacggatacacagtggtgagaaatcagagtctatctcagtctaa

SEQ ID NO: 4 - DNA, 20 bp, Artificial Sequence
  primer sequence of Zkscan8
cggaggaaagtcggaaacca

SEQ ID NO: 5 - DNA, 20 bp, Artificial Sequence
  primer sequence of Zkscan8
cttcccgtggaccaagagtc

SEQ ID NO: 6 - DNA, 20 bp, Artificial Sequence
  primer sequence of PPAR gamma 2
ttggtgactttatggagccc

SEQ ID NO: 7 - DNA, 20 bp, Artificial Sequence
  primer sequence of PPAR gamma 2
catgtctgtctccgtcttct

SEQ ID NO: 8 - DNA, 20 bp, Artificial Sequence
  primer sequence of aP2
aagaagtaggagtgggcttt

SEQ ID NO: 9 - DNA, 20 bp, Artificial Sequence
  primer sequence of aP2
ccaccaccagtttatcatcc

SEQ ID NO: 10 - DNA, 20 bp, Artificial Sequence
  primer sequence of Osteopontin
gagacccttccaagtaagtc

SEQ ID NO: 11 - DNA, 20 bp, Artificial Sequence
  primer sequence of Osteopontin
gatgtcctcgtctgtagcat

SEQ ID NO: 12 - DNA, 20 bp, Artificial Sequence
  primer sequence of ALP
tggagcttcagaagctcaac

SEQ ID NO: 13 - DNA, 20 bp, Artificial Sequence
  primer sequence of ALP
atctcgttgtctgagtacca

SEQ ID NO: 14 - DNA, 20 bp, Artificial Sequence
  primer sequence of Sox6
aacatgtggcctcccatctg

SEQ ID NO: 15 - DNA, 20 bp, Artificial Sequence
  primer sequence of Sox6
tcagtgtgtccaccacatcg

SEQ ID NO: 16 - DNA, 20 bp, Artificial Sequence
  primer sequence of Aggrecan
tcaggagggctggaacaagt

SEQ ID NO: 17 - DNA, 20 bp, Artificial Sequence
  primer sequence of Aggrecan
ggaggtggtaattgcaggga

SEQ ID NO: 18 - DNA, 20 bp, Artificial Sequence
  primer sequence of Mkx
ggccacgaacactaccatga

SEQ ID NO: 19 - DNA, 20 bp, Artificial Sequence
  primer sequence of Mkx
agctgcgctttcacccttat

SEQ ID NO: 20 - DNA, 20 bp, Artificial Sequence
  primer sequence of Egr-1
ccagtggagtcctgtgatcg

SEQ ID NO: 21 - DNA, 20 bp, Artificial Sequence
  primer sequence of Egr-1
tcgctcctggcaaactttct

SEQ ID NO: 22 - DNA, 20 bp, Artificial Sequence
  primer sequence of Egr-2
tcttcctctctggcctaccc

SEQ ID NO: 23 - DNA, 20 bp, Artificial Sequence
  primer sequence of Egr-2
gtctgttggggtacttgcga

SEQ ID NO: 24 - DNA, 20 bp, Artificial Sequence
  primer sequence of COL1a1
agtggtttggatggtgccaa

SEQ ID NO: 25 - DNA, 20 bp, Artificial Sequence
  primer sequence of COL1a1
gcaccatcatttccacgagc

SEQ ID NO: 26 - DNA, 19 bp, Artificial Sequence
  primer sequence of COL3a1
cttctctccagccgagctt

SEQ ID NO: 27 - DNA, 20 bp, Artificial Sequence
  primer sequence of COL3a1
ccagtgtgtttcgtgcaacc

SEQ ID NO: 28 - DNA, 20 bp, Artificial Sequence
  primer sequence of Desmin
gaggaaatccggcacctcaa

SEQ ID NO: 29 - DNA, 21 bp, Artificial Sequence
  primer sequence of Desmin
catccccgtgtctcgatggtc

SEQ ID NO: 30 - DNA, 20 bp, Artificial Sequence
  primer sequence of NEFL
ctggaaatcgaagcatgccg

SEQ ID NO: 31 - DNA, 20 bp, Artificial Sequence
  primer sequence of NEFL
gcgggtggacatcagatagg

SEQ ID NO: 32 - DNA, 22 bp, Artificial Sequence
  primer sequence of GAPDH
aaatcccatcaccatcttccag

SEQ ID NO: 33 - DNA, 21 bp, Artificial Sequence
  primer sequence of GAPDH
catgagtccttccacgatacc